European Patent Application EP 4 578 953 A1, published July 2, 2025. Title: Methods for producing compositions, oligosaccharide-containing compositions obtained thereby, and use thereof. Applicant: MEIJI CO., LTD. The sequence listing filed with the application follows.

SEQUENCE LISTING (21 sequences)

SEQ ID NO: 1 - protein, 1075 aa, Liquorilactobacillus satsumensis
MEQLEMEAQAQFDEVHAKIRRTRGSGQQPHEHKHIGKRQQRENSTKTVFAGNSPDVPIIFGGRYVEVSGTWFYLDSHGNKLKGLNKVDGNLQYFDQTSGAQLKGEFEKVGGVTYYFDKSSGNAIPYVLTVGSQKTAYQSDGTPAASGFFTAQDGHIYYFNSIGSYVTGLQTIAGATYYFDEDGYLAKDTLETVNGKSYYSDVLTGQVVELVAQTIPSQPSSAKAIAAFAAHNVAYSYTAKSFENIDGYLTADSWYRPTEILSDGQRWVKTTETDFRPLLMAWWPSKAIQADYLNYLVAQGIVQSKQQFSANDSFRVLASAAQNVQIAFEKNLMLTATANWLRQLLHNFIKTEEIWNKSSEDVSSDGLQSLQGGFLAYQNSKRTPKANSKARILGYVPSYIKNNENKGSEFLLANDIDNSNPIVQAEELNWLHYLMNFGTITANDATANFDGIRVDAVDNVDADLLQIAAEYFKNAYHVDQNDQAANAHLSILEDWGSDDPQYIFDQGANQLTMDDYVVGQMNYSLESGPEANDKMARFLQWYLINRANDSTENTAIPNYTFVRAHDSNSQDQIQKAVQAATGGEYGAFTWAQLQQGLELYYADQASTTKEYNRYNMPSAYAMLLTNKDSIPRVYYGDMYLEGGQYLANKTIYYDTIANLLKTRIKYVAGGQTMSVDSNDILTSVRFGKGAMTAADQGTAETRTEGIGVVIGNNTALELKDGAQVILHMGAAHRKQAYRAAVLTTETGVINYPTDEGAPLAYTNDAGDLIFTNQNLVVNGQTEANTSVQGYANPAVTGYLAVWVPAGASATQDARTTATTLPQADGKIFHSNAALDSNVIFEGFSNFISYPETHDENANVVIAKKTALFKALGITSFELAPQYRSSGDHTFLDATIDNGYAFTDRYDLGFGTPTKYGTVDDLRNALKALHAAGIQAIADWVPDQLYNLPTKELVTVNRTDERGNQLADSKIHRLLYVANTIGGGEYQKQYGGAFLSLLETEYPDLFTAIQASTHKPLDPSVKITSWSAKYLNGTNILGRGIGYVLRDAHNSYFFVGEDSPVAQRLLPETLIAEPAE

SEQ ID NO: 2 - protein, 1483 aa, Liquorilactobacillus satsumensis
VGDDGQVKKNFTAVINGQVLYFDKDTGALASNDKQYTNGLVNIGNQHNAAYSTTTDSFTQVDGYLTAESWYRPKDILKNGTTWTASTTTDFRPLLMTWWPDKNTQLAYLEYMQKAGLLEDSVSLSNTSTQAFLTNEALSAQANIEKKISLAGNTDWLKTEITQFVDAQPNWNIKSESKGTDHLQGGALLYVNSSLTPAANSDSRLLNRTPKNQEGQIPSTENQGGYEMLLANDVDNSNPVVQAEQLNWLYYMMNIGTIAGNDSSANFDGYRVDAVDNVDADLLQIASDYFKDAYGTNQSDSNANNHLSILEDWESSDADYVKEHGNNQLTMDFHSHLAVKYSLNMPTNERSGLEPELTYSLVNRTGDNSTENVAQPNYSFIRAHDSEVQTVIAQIIKDKINPDSDGLTVTSAEIAQAFKIYNQDELQADKKYTAYNIPSSYALLLTNKDTVPRVYYGDLFTDDGQYMATHSPYYDALTALLKARVKYVSGGQNMGIQYVQGDNSMASSSYRGVLTSVRYGKDALSASSTGDANTRTQGMAVVLSNNPDLKLSQSDQVVVNMGAAHRNQAYRALLLTTKEGLKVYSADDGAPVVYTNDLGQLIFKRDSIFGVSDPQVSGYLAAWVPVGASSTQDARTASSTATSTDGKTYHSNAALDSQVIFEGFSNFQAMPTQTAEYTNVKIAQNAQLFKDLGITSFELAPQYRSSTDASFLDSVVQNGYAFTDRYDVGYNTPTKYGTVAQLLSAIKALHAQGIQAINDWVPDQIYNLPGEEIVTAVRTNGSGVSNQDSVINNTLYDSHTVGGGQYQAMYGGAFLDRIKQLYPDLFETKQISTGQPMNPNEKITEWSAKYFNGSNIQGRGAWYVLKDWATNKYFSVSSNNSFLPKQLQGKKASTGFVVDSKNRTKFYSTSGYQAKNTFIQDGDNWYYFDNNGYMVTGADKINGYNYYFLPNGIELQDAYFADGTKEYYYSKSGKQILDQYYQDSNGNWRYFFKDGTMAKGLTQITAVNGQTVTQYFDTDGIQVKGNAAKDSDGKLRYFDGITGNMVVNSFGELPDGSWLYLDENGVAVTGKQNINGQTMYFNADGRQVKNDFGELADGSWLYLNSDGVAVIGEQVINGKTLYFNADGKQVKNDFKQLADGSWLYLNSDGVAVTGKQVINGKTLYFNADGKQVKNDFKQLADGSWLYLNGDGVAVTGEQVINGKTLYFNADGKQVKNDFKQLADGSWLYLNGDGVAVKGKQVINGKTLYFNADGKQVKNDFKQLADGDGVAVTGEQVINGKTLYFNADGRQVKNDFKQLADGSWVYLNGDGVAVTGKQVINGKTLYFNADGRQVKNDFKQLADGSWLYLNSDGVAVTGEQVINGKTLYFNADGKQVKNDFKELANGSWLYLDGNGVAVTGKQVINGQTMYFNADGTQVKNDFGELADGSWLYLGADGVAVTGKQTIRGQKLYFRSNGIQVKGGSVLEEDGQWHTYDLNSGEELR

SEQ ID NO: 3 - protein, 1715 aa, Liquorilactobacillus satsumensis
VKETKTHYKMYKKGKNWVFAAITVTTIGYGLLGINSEHAAAASNDATVTAGSETVSSNTSSSTQAEKTSEQAKSSAKVTTSTSSSASDSDSKTNSSSSTQKVSNSQSNTTTSASHVSSTEAAVSSSAKSSTNADKTSSSQASSQSSQSSSQASSTAQSSSAQPNSSSQSNSSSQSETNKDTATKDPLVDTETNLQNGHYVANNDTWTYVDDQGNVVKGLKKIDGNVQYFDPQTGVQIKGEYVTVGKQTYYFDPHSGNAIAYSKTNGDTFAAYNADSSVAQQGFFTDQNGNTYYLESSTQYKIGLQEINKVTYYFGEDGILRKNTTQTIDGRLYCFASDGSAKLLPQDKLTESQASAKEVADFAAHNVAKSYDAQSFENTNGYLTADSWYVPKYILSNGQQWVASSASDFRPLLMAWWPSKQVQADYLNYMAGRGVVAATKTYSANDTSLELNGAVEAVQATIERALKITGNVTWLRDVMSKFVKEETIWNKESEDVQYYGLQLQGGFLAYQNSSLTPWANSDYRKLGFTPGYLDGKSNKDAEFLLANDIDNSNPTVQAEQLNWLYYLTNFGTITANNANANFDGIRVDAVDNVDADLLQIAADYFNAAYGTNQSDASANKHLSILEDWGMNDPAYISEHGASQLTMDNYMGVQLNSSLTNAQGQNDKMARFVQWFLINRTNDDTEDTAIPNYSFVRAHDSNSQDQVRQAIQDATGKPYGQFTWADLEKGLELFYKDQDSTVKKYNKYNIPSAYAMLLTNKDTVPRVFYGDMYSEGGQYLSQKTIYYDTLTNLLKSRIKYVGGGQTMAVDQNDVLTSVRFGKGALNVTDQGTSETRTEGVGVIIANNTDLKLKDGEQVVLHMGAAHKNQAFRAAVLTTSTGLVNYENDTAAPVVYTDNNGDLIFTNKDLVVAGQTVANTAIQGVATPQVTGYLAVWVPVGAAAEQDARTAASDQTSTDGKVFHSNAALDSNVIFEGFSNFISYPQERSQYANIVIAQNAAAFKQLGITSFELAPQYRSSSDGSFLDSMIDNGYAFTDRYDLGFGTPTKYGTAADLRNAIAALHANGIQAIADWVPDQIYALPGQETVTVTRTDDHGNWISDSSIHDSLYVANTIGGGEYQNKYGGAFLAELQQKYPELFTKNQAVTGVPIDGSTKIKEWSAKYLNATNILGRGSEYVLKSNDNGEYFYVGTERTAFLPAVLVAQNERAEYAAGDSSQARYYAQLEDTAGHWYLIDPTTGTKQTGFQKIIDQNKVVYYNNAGQMQYGQQKINGQWYLFDSYDGAMKTGLQSIKGQNKTVYYNDKGQMQYGQQKINDSWYLFDGYTGAMKTGWQYLAAQNKLVHYATNGQMQHGQQKIDGRWYYFDTVTGSQKFGLQYLADQNKTVDYGSQGWMQYGQQKIDGQWYLFDSYDGAMKTGLQYINGQNKTVYYNAKGQMQYGQQKIGDDWYLFDGYTGAMKTGWQYLASQNKLVHYASNGQMQYGQQKIDGRWYYFDTVTGSQKFGLQYLADQHKTVFYGNQGQMQYGQQKIDGQWYLFDSYDGAMKTGLQYINGQNKTVYYNAKGQMQYGQQKVGDNWYLFDGYTGAMKTGWQYLANQNKLVHYASNGQMQYGQQKINGRWYYFDTLTGAQKFGLQYLADQNKTVDYGSQGWMQYGQQKIGNDWYLFDDYDGAMKTGWQYLAAQNKTVYYNESGKMVYGQQKIDGKVYNFDTVTGALKK

SEQ ID NO: 4 - protein, 1417 aa, Liquorilactobacillus satsumensis
MARLDKRKLVLNKPERYLVTAEIALALGLGLNCTFGAHVHADTVMTTKQVQVTEKTTSDSPDSAEKTGVTTASTKDTVQSGTATTTQTPETTQTPNTGAQLGAPLIENTTQTAATSSTPTATPNTATQTPATSSTPTATPDTTTQTPATSSTPTATPDTTTQTPATNSTPTATPDTTTQTAATSSTPTATSSTATQTADLTVTTASSTGDTHIQTIEGKTYFVGDDGKVKKNFTAVVNGQVMYFDNETGALTSNEKQYTNGLVNIGNEHNAAYSASADNFTQVNGYLTAESWYRPKDILKGGTTWTASTATDFRPLLMTWWPDKTTQLAYLEYMQKNGLLGTDVKLASNDNQQLLTDEAFKVQQNIESKISSVGSTDWLKNSITQFVDAQPNWNITSESKGTDHLQGGALLYVNSSLTPAANSDSRLLNRTPKNQEGQIPSTENQGGYEMLLANDVDNSNPVVQAEQLNWLYYMMNIGTIAGNDSSANFDGYRVDAVDNVDADLLQIAGDYFKAAYGTNQNDANANRHLSILEDWESSDAAYVKEHGNNQLTMDFPIHLALKYSLNTPLGQRSNLEANLTTSLVNRTNDNAAESGAQPNYSFIRAHDSEVQTVIAQIIKDHINPNSDGLTVTPEEIAQAFKIYNQDELQADKKYTAYNIPSSYALLLTNKDTVPRVYYGDLFTDDGQYMAAHSPYYDALTALLKARVKYVSGGQNMGVEYVQGDSTMDSGSYRGVLTSVRYGKDALSASSTGDADTRTQGIAVVLSNNPDLKLSQSDQVVVNMGVAHRNQAYRALLLTTKEGLKVYSADDGAPVVYTNDLGQLIFKRDSIFGVSDPQVSGYLAAWVPVGASSTQDARTASSTAVSTDGSTFHSNAALDSQVIFEGFSNFQAMPTQTAEYTNVKIAQNAQLFKDLGITSFELAPQYRSSTDASFLDSVVQNGYAFTDRYDVGYNTPTKYGTVAQLLSAIKALHAQGIQAINDWVPDQIYNLPGEEIVTAERTNSAGIYDQDSAINNTLYDSHTVGGGQYQAMYGGAFLDKIKQLYPDLFKTKQISTGQSMNPNEKITEWSAKYFNGSNIQGRGAWYVLKDWATNKYFSVSSNNSFLPNQLLAGKASTGFVTENDKTTFYSTSGYQAKGTFIQDGNNWYYFDNDGYMVTGANKINGYNYYFLPNGIELRDAYLSDGNKSYYYNKAGRQVADRYYLLADGNWRYFFKDGTMAKGLTQITAVNGETVTQYFDSEGIQVKGKAVIDSSNNIRYFAENTGDMVIDGFGKDSDGSWLYLDHQGVAVTGKQVINGQTLYFNADGRQVKNDFKELADGSWLYLDQNGVAVTGKQVINGQTLYFNADGRQVKDDFKELPDGSWLYLDQNGVAVTGKQTIRGQHLYFKADGIQVKGDAVLEADGKLHYYDPDSGEEWL

SEQ ID NO: 5 - protein, 1290 aa, Leuconostoc meseteroides
MPNVKHVDGKVYFYGDDGQPKKNFTTIIDGKPYYFDKDTGALSNNDKQYVSELFSIGNKHNAVYNTSSDNFTQLEGHLTASSWYRPKDILKNGKRWAPSTVTDFRPLLMAWWPDKSTQVTYLNYMKDQGLLSGTHHFSDNENMRTLTAAAMQAQVNIEKKIGQLGNTDWLKTAMTQYIDAQPNWNIDSEAKGDDHLQGGALLYTNSDMSPKANSDYRKLSRTPKNQKGQIADKYKQGGFELLLANDVDNSNPVVQAEQLNWLHYMMNIGSILQNDDQANFDGYRVDAVDNVDADLLQIAGEYAKAAYGVDKMTRERINIYQFWKTGEMKIQTMSKHMATSKLSMDFPLHLAIKYALNMPNDKRSGLEPTREHSLVKRITDDKENVAQPNYSFIRAHDSEVQTIIADIIKDKINPASTGLDSTVTLDQIKQAFDIYNADELKADKVYTPYNIPASYALLLTNKDTIPRVYYGDMFTDDGQYMAKQSPYYQAIDALLKARIKYAAGGQTMKMNYFPDEQSVMTSVRYGKGAMTASDSGNQETRYQGIGLVVNNRPDLKLSDKDEVKMDMGAAHKNQDYRPVLLTTKSGLKVYSTDANAPVVRTDANGQLTFKADMVYGVNDPQVSGYIAAWVPVGASENQDARTKSETTQSTDGSVYHSNAALDSQVIYEGFSNFQDFPTTPDEFTNIKIAQNVNLFKDWGITSFEMAPQYRASSDKSFLDAIVQNGYAFTDRYDIGYNTPTKYGTADNLLDALRALHGQGIQAINDWVPDQIYNLPDEQLVTAIRTDGSGDHTYGSVIDHTLYASKTVAGGIYQQQYGGAFLEQLKTQYPQLFQQKQISTDQPMNPDIQIKSWEAKYFNGSNIQGRGAWYVLKDWGTQQYFNVSDAQTFLPKQLLGEKAKTGFVTRGKETSFYSTSGYQAKSAFICDNGNWYYFDDKGKMVVGNQVINGINYYFLPNGIELQDAYLVHDGMYYYYNNIGKQLHNTYYQDKQKNFHYFFEDGHMAQGIVTIIQSDGTPVTQYFDENGKQQKGVAVKGSDGHLHYFDGASGNMLFKSWGRLADGSWLYVDEKGNAVTGKQTINNQTVYFNDDGRQIKNNFKELADGSWLYLNNKGVAVTGEQIINGQTLYFGNDGRQFKGTTHINATGESRYYDPDSGNMITDRFERVGDNQWAYFGYDGVAVTGDRIIKGQKLYFNQNGIQMKGHLRLENGIMRYYDADTGELVRNRFVLLSDGSWVYFGQDGVPVTGVQVINGQTLYFDADGRQVKGQQRVIGNQRYWMDKDSGEMKKITY

SEQ ID NO: 6 - protein, 1527 aa, Leuconostoc citreum
MEQQETVTRKKLYKSGKSWVAAATAFAVMGVSAVTTVSDTHKTPVGTTQSQQALTGQTGQDKPTTKEVIDKKEPVPESTTNNDSKSVHASGKNIDQQNELNKNTATENNKKTQDQNTATTPDTKESNKAVSDDQKITVQDDRNIALSKNLVDNKDAISTVITGGRYEQQDGHFVYLDQSGKKVIGLQNINGNVQYFDENGAQVKGDFRPGKEKNKVYFDKNTGNAIAYISNVHGVINGVDATGKQIKDNFLTDEKGNTYYFDSQGNMLKGLQTLDGKQYYFDEEGLLKKNYAATFNNQVIYFDSVTGIGKTALEYQFSQGLTDQKSDFTAHNAANSYDAKSFDNIQGFLTADSWYQPKDILKGGKTWVASTEDDKRPLLMTWWPDKQTQANYINYMSKTFATNDGIQYDATTNQSTLNLATQNIQVLIEQRIAQANSIQWLKNEMSNFIKEQFNWSKKSENIDYGGLQFQGGFLKYNNTPLASDTNSAFRLLNRVLFNRDGNSNVKGSEFLLANDVDNSNPVVQAEQLNWLHYLMNFGTITANDPDANFDSIRVDAVDNVDADLLDIARDYFNAVYKVNQSDVNANKHISILEDWSGLDPNEVVKNGNPQLTLNTGVQNSLLNALTKGPNNRWGIDSLIDKSTMRYPDKDGKILIPNYSFVRAHDSEVQGIIGKILTDHTSAESGNKFTKDQLKQALDYYYADQDKTVKEYSHYNMASAYAALLTNKNTIPRVYYGDMYKDNDSYMTSKTNEFDSIDALLKARIKYVSGNQEMGVDTKHQDVLTSVRNGNSRTEGIGVIISNNPNLNLGSDKITLSMGVNHANQMYRPLLLATDNGIDVYITDSSTTIRETTDGNGNLEFSSNYIKGYGINNSKVSGYLAVWVPVGADDKQDARVATSQNKTTDGSVFHANDALDTNVIYEGFSNFQQTPNLVDKDQRTNVIIAKEAKNGTFSNWGITSFQMPPQYRSSHDGTFVDSTIDNGYAFTDRYDLGFNNDDGTENPTKYGTVEDLRNAIKALHSKSIQAMADWVPDQIYNLSGQQVTSVTRVNEKGETWPNADIENVLYVVDTVGGGKYQAEYGGKYLGELQQKYPDLFTKPQITTGVPMDANTRIKEWSAKYFNGTNILGRGAYYVLKDWASNQYFNVNKADEAFLPLQLMNQDAKTGFVIDAVGVKYYSISGYQAKNSFIQDDNHNWYYFDNNGYMVRPENGKSGLVQMKVTNADGTVRESLDSSNKDGRYYYFMPNGMEIRNGFVKDIDGKSYYFNSVGEMLTNQYVFDASGNAYHLNSDGTMSTGLVLAGYNNVYHYYGLNGVQVKGKVAYDKNTNKWYSFDANSGDSQAFTDRPNNTQDFITIDTSSTLGVNADYTAYITSSVRQDGLFANAPYGVITKDQTGNDIKWEFINKDTKQYEGQQVQVTRQYTDSKGVSWNLITFAGGDLQGQKLWVDSRALTMTPFKTMNQISFISYANRNDGLFLNAPYQVKGYQLAGMSNQYKGQQVTIAGVANVSGKDWSLISFNGTQYGLIVSH

SEQ ID NO: 7 - protein, 1476 aa, Streptococcus mutans
MDKKVRYKLRKVKKRWVTVSVASAVMTLTTLSGGLVKADSNESKSQISNDSNTSVVTANEESNVTTEVTSKQEAASSQTNHTVTTISSSTSVVNPKEVVSNPYTVGETASNGEKLQNQTTTVDKTSEAAANNISKQTTEADTDVIDDSNAANLQILEKLPNVKEIDGKYYYYDNNGKVRTNFTLIADGKILHFDETGAYTDTSIDTVNKDIVTTRSNLYKKYNQVYDRSAQSFEHVDHYLTAESWYRPKYILKDGKTWTQSTEKDFRPLLMTWWPSQETQRQYVNYMNAQLGINKTYDDTSNQLQLNIAAATIQAKIEAKITTLKNTDWLRQTISAFVKTQSAWNSDSEKPFDDHLQNGAVLYDNEGKLTPYANSNYRILNRTPTNQTGKKDPRYTADNTIGGYEFLLANDVDNSNPVVQAEQLNWLHFLMNFGNIYANDPDANFDSIRVDAVDNVDADLLQIAGDYLKAAKGIHKNDKAANDHLSILEAWSDNDTPYLHDDGDNMINMDNKLRLSLLFSLAKPLNQRSGMNPLITNSLVNRTDDNAETAAVPSYSFIRAHDSEVQDLIRDIIKAEINPNVVGYSFTMEEIKKAFEIYNKDLLATEKKYTHYNTALSYALLLTNKSSVPRVYYGDMFTDDGQYMAHKTINYEAIETLLKARIKYVSGGQAMRNQQVGNSEIITSVRYGKGALKATDTGDRTTRTSGVAVIEGNNPSLRLKASDRVVVNMGAAHKNQAYRPLLLTTDNGIKAYHSDQEAAGLVRYTNDRGELIFTAADIKGYANPQVSGYLGVWVPVGAAADQDVRVAASTAPSTDGKSVHQNAALDSRVMFEGFSNFQAFATKKEEYTNVVIAKNVDKFAEWGVTDFEMAPQYVSSTDGSFLDSVIQNGYAFTDRYDLGISKPNKYGTADDLVKAIKALHSKGIKVMADWVPDQMYAFPEKEVVTATRVDKFGKPVEGSQIKSVLYVADSKSSGKDQQAKYGGAFLEELQAKYPELFARKQISTGVPMDPSVKIKQWSAKYFNGTNILGRGAGYVLKDQATNTYFNISDNKEINFLPKTLLNQDSQVGFSYDGKGYVYYSTSGYQAKNTFISEGDKWYYFDNNGYMVTGAQSINGVNYYFLSNGLQLRDAILKNEDGTYAYYGNDGRRYENGYYQFMSGVWRHFNNGEMSVGLTVIDGQVQYFDEMGYQAKGKFVTTADGKIRYFDKQSGNMYRNRFIENEEGKWLYLGEDGAAVTGSQTINGQHLYFRANGVQVKGEFVTDRYGRISYYDSNSGDQIRNRFVRNAQGQWFYFDNNGYAVTGARTINGQHLYFRANGVQVKGEFVTDRHGRISYYDGNSGDQIRNRFVRNAQGQWFYFDNNGYAVTGARTINGQHLYFRANGVQVKGEFVTDRYGRISYYDSNSGDQIRNRFVRNAQGQWFYFDNNGYAVTGARTINGQHLYFRANGVQVKGEFVTDRYGRISYYDANSGERVRIN

SEQ ID NO: 8 - protein, 1772 aa, Limosilactobacillus reuteri
MEIKKHFKLYKSGKQWVTAAVATVAVSTALLYGGVAHADQQVQSSTTQEQTSTVNADTTKTVNLDTNTDQPAQTTDKNQVANDTTTNQSKTDSTSTTVKNPTFIPVSTLSSSDNEKQSQNYNKPDNGNYGNVDAAYFNNNQLHISGWHATNASQGTDSRQVIVRDITTKTELGRTNVTNNVLRPDVKNVHNVYNADNSGFDVNINIDFSKMKDYRDSIEIVSRYSGNGKSVDWWSQPITFDKNNYAYLDTFEVKNGELHATGWNATNKAINYNHHFVILFDRTNGKEVTRQEVRDGQSRPDVAKVYPQVVGANNSGFDVTFNIGDLDYTHQYQILSRYSNADNGEGDYVTYWFAPQSIAPANQSNQGYLDSFDISKNGEVTVTGWNATDLSELQTNHYVILFDQTAGQQVASAKVDLISRPDVAKAYPTVKTAETSGFKVTFKVSNLQPGHQYSVVSRFSADENGNGNDKRHTDYWYSPVTLNQTASNIDTITMTSNGLHITGWMASDNSINEATPYAIILNNGREVTRQKLTLIARPDVAAVYPSLYNSAVSGFDTTIKLTNAQYQALNGQLQVLLRFSKAVDGNPNGTNTVTDQFSKNYATTGGNFDYVKVNGNQIEFSGWHATNQSNDKNSQWIIVLVNGKEVKRQLVNDTKDGAAGFNRNDVYKVNPAIENSIMSGFQGIITLPVTVKDENVQLVHRFSNDAKTGEGNYVDFWSEVMSVKDSFQKGNGPLNQFGLQTINGQQYYIDPTTGQPRKNFLLQNGNDWIYFDKDTGAGTNALKLQFDKGTISADEQYRRGNEAYSYDDKSIENVNGYLTADTWYRPKQILKDGTTWTDSKETDMRPILMVWWPNTVTQAYYLNYMKQYGNLLPASLPSFSTDADSAELNHYSELVQQNIEKRISETGSTDWLRTLMHEFVTKNSMWNKDSENVDYGGLQLQGGFLKYVNSDLTKYANSDWRLMNRTATNIDGKNYGGAEFLLANDIDNSNPVVQAEELNWLYYLMNFGTITGNNPEANFDGIRVDAVDNVDVDLLSIARDYFNAAYNMEQSDASANKHINILEDWGWDDPAYVNKIGNPQLTMDDRLRNAIMDTLSGAPDKNQALNKLITQSLVNRANDNTENAVIPSYNFVRAHDSNAQDQIRQAIQAATGKPYGEFNLDDEKKGMEAYINDQNSTNKKWNLYNMPSAYTILLTNKDSVPRVYYGDLYQDGGQYMEHKTRYFDTITNLLKTRVKYVAGGQTMSVDKNGILTNVRFGKGAMNATDTGTDETRTEGIGVVISNNTNLKLNDGESVVLHMGAAHKNQKYRAVILTTEDGVKNYTNDTDAPVAYTDANGDLHFTNTNLDGQQYTAVRGYANPDVTGYLAVWVPAGAADDQDARTAPSDEAHTTKTAYRSNAALDSNVIYEGFSNFIYWPTTESERTNVRIAQNADLFKSWGITTFELAPQYNSSKDGTFLDSIIDNGYAFTDRYDLGMSTPNKYGSDEDLRNALQALHKAGLQAIADWVPDQIYNLPGKEAVTVTRSDDHGTTWEVSPIKNVVYITNTIGGGEYQKKYGGEFLDTLQKEYPQLFSQVYPVTQTTIDPSVKIKEWSAKYFNGTNILHRGAGYVLRSNDGKYYNLGTSTQQFLPSQLSVQDNEGYGFVKEGNNYHYYDENKQMVKDAFIQDSVGNWYYFDKNGNMVANQSPVEISSNGASGTYLFLNNGTSFRSGLVKTDAGTYYYDGDGRMVRNQTVSDGAMTYVLDENGKLVSESFDSSATEAHPLKPGDLNGQK

SEQ ID NO: 9 - protein, 18 aa, Leuconostoc meseteroides
DGIRVDAVDNVDADLLQI

SEQ ID NO: 10 - protein, 18 aa, Limosilactobacillus reuteri
DSVRVDAPDNIDADLMNI

SEQ ID NO: 11 - protein, 18 aa, Liquorilactobacillus satsumensis
DGYRVDAVDNVDADLLQI

SEQ ID NO: 12 - protein, 12 aa, Leuconostoc meseteroides
HLSILEDWSHND

SEQ ID NO: 13 - protein, 12 aa, Limosilactobacillus reuteri
HINILEDWNHAD

SEQ ID NO: 14 - protein, 12 aa, Liquorilactobacillus satsumensis
HLSILEDWGSDD

SEQ ID NO: 15 - protein, 12 aa, Liquorilactobacillus satsumensis
HLSILEDWGMND

SEQ ID NO: 16 - protein, 12 aa, Liquorilactobacillus satsumensis
HLSILEDWESSD

SEQ ID NO: 17 - protein, 15 aa, Leuconostoc meseteroides
YSFVRAHDSEVQTVI

SEQ ID NO: 18 - protein, 15 aa, Limosilactobacillus reuteri
YSFVRAHDNNSQDQI

SEQ ID NO: 19 - protein, 15 aa, Liquorilactobacillus satsumensis
YTFVRAHDSNSQDQI

SEQ ID NO: 20 - protein, 15 aa, Liquorilactobacillus satsumensis
YSFVRAHDSNSQDQV

SEQ ID NO: 21 - protein, 15 aa, Liquorilactobacillus satsumensis
YSFIRAHDSEVQTVI